European Patent Application EP 4 245 771 A1, published September 20, 2023. Title: A novel calreticulin-specific binding protein having human fibronectin III domain scaffold and use thereof. Applicant: INDUSTRY FOUNDATION OF CHONNAM NATIONAL UNIVERSITY. The sequence listing filed with the application follows.

SEQUENCE LISTING (21 sequences)

SEQ ID NO: 1 - DNA, 318 bp, Artificial Sequence
  CRT1
atggctagcgtttctgatgttccgagggacctggaagttgttgctgcgacccccaccagcctactgatcagctgggatgctcctgctgtcacagtgagatattacaggatcacttacggagaaacaggaggaaatagccctgtccaggagttcactgtgcctgggagcaagtctacagctaccatcagcggccttaaacctggagttgattataccatcactgtgtatgctgtcactggtcaaccaatgtatggtcaaccaatgtatccaatttccattaattaccgaacaggatcccaccatcaccatcatcactga

SEQ ID NO: 2 - DNA, 309 bp, Artificial Sequence
  CRT2
atggctagcgtttctgatgttccgagggacctggaagttgttgctgcgacccccaccagcctactgatcagctgggatgctcctgctgtcacagtgagatattacaggatcacttacggagaaacaggaggaaatagccctgtccaggagttcactgtgcctgggagcaagtctacagctaccatcagcggccttaaacctggagttgattataccatcactgtgtatgctgtcactaaattaggtttttttaaaagaccaatttccattaattaccgaacaggatcccaccatcaccatcatcactga

SEQ ID NO: 3 - DNA, 315 bp, Artificial Sequence
  CRT3
atggctagcgtttctgatgttccgagggacctggaagttgttgctgcgacccccaccagcctactgatcagctggaaattaggtttttttaaaagatattacaggatcacttacggagaaacaggaggaaatagccctgtccaggagttcactgtgcctgggagcaagtctacagctaccatcagcggccttaaacctggagttgattataccatcactgtgtatgctgtcactggtcaaccaatgtatggtcaaccaatgtatccaatttccattaattaccgaacaggatcccaccatcaccatcatcactga

SEQ ID NO: 4 - DNA, 315 bp, Artificial Sequence
  CRT4
atggctagcgtttctgatgttccgagggacctggaagttgttgctgcgacccccaccagcctactgatcagctggggtcaaccaatgtatggtcaaccaatgtattattacaggatcacttacggagaaacaggaggaaatagccctgtccaggagttcactgtgcctgggagcaagtctacagctaccatcagcggccttaaacctggagttgattataccatcactgtgtatgctgtcactaaattaggtttttttaaaagaccaatttccattaattaccgaacaggatcccaccatcaccatcatcactga

SEQ ID NO: 5 - DNA, 324 bp, Artificial Sequence
  CRT5
atggctagcgtttctgatgttccgagggacctggaagttgttgctgcgacccccaccagcctactgatcagctggggtcaaccaatgtatggtcaaccaatgtattattacaggatcacttacggagaaacaggaggaaatagccctgtccaggagttcactgtgcctgggagcaagtctacagctaccatcagcggccttaaacctggagttgattataccatcactgtgtatgctgtcactggccgtggagacagccccgcaagcagcaagccaatttccattaattaccgaacaggatcccaccatcaccatcatcactga

SEQ ID NO: 6 - DNA, 315 bp, Artificial Sequence
  CRT6
atggctagcgtttctgatgttccgagggacctggaagttgttgctgcgacccccaccagcctactgatcagctggaaattaggtttttttaaaagatattacaggatcacttacggagaaacaggaggaaatagccctgtccaggagttcactgtgcctgggagcaagtctacagctaccatcagcggccttaaacctggagttgattataccatcactgtgtatgctgtcactggccgtggagacagccccgcaagcagcaagccaatttccattaattaccgaacaggatcccaccatcaccatcatcactga

SEQ ID NO: 7 - protein, 105 aa, Artificial Sequence
  CRT1
MASVSDVPRDLEVVAATPTSLLISWDAPAVTVRYYRITYGETGGNSPVQEFTVPGSKSTATISGLKPGVDYTITVYAVTGQPMYGQPMYPISINYRTGSHHHHHH

SEQ ID NO: 8 - protein, 102 aa, Artificial Sequence
  CRT2
MASVSDVPRDLEVVAATPTSLLISWDAPAVTVRYYRITYGETGGNSPVQEFTVPGSKSTATISGLKPGVDYTITVYAVTKLGFFKRPISINYRTGSHHHHHH

SEQ ID NO: 9 - protein, 104 aa, Artificial Sequence
  CRT3
MASVSDVPRDLEVVAATPTSLLISWKLGFFKRYYRITYGETGGNSPVQEFTVPGSKSTATISGLKPGVDYTITVYAVTGQPMYGQPMYPISINYRTGSHHHHHH

SEQ ID NO: 10 - protein, 104 aa, Artificial Sequence
  CRT4
MASVSDVPRDLEVVAATPTSLLISWGQPMYGQPMYYYRITYGETGGNSPVQEFTVPGSKSTATISGLKPGVDYTITVYAVTKLGFFKRPISINYRTGSHHHHHH

SEQ ID NO: 11 - protein, 107 aa, Artificial Sequence
  CRT5
MASVSDVPRDLEVVAATPTSLLISWGQPMYGQPMYYYRITYGETGGNSPVQEFTVPGSKSTATISGLKPGVDYTITVYAVTGRGDSPASSKPISINYRTGSHHHHHH

SEQ ID NO: 12 - protein, 104 aa, Artificial Sequence
  CRT6
MASVSDVPRDLEVVAATPTSLLISWKLGFFKRYYRITYGETGGNSPVQEFTVPGSKSTATISGLKPGVDYTITVYAVTGRGDSPASSKPISINYRTGSHHHHHH

SEQ ID NO: 13 - DNA, 318 bp, Artificial Sequence
  DGR Scrambled monobody
atggctagcgtttctgatgttccgagggacctggaagttgttgctgcgacccccaccagcctactgatcagctgggatgctcctgctgtcacagtgagatattacaggatcacttacggagaaacaggaggaaatagccctgtccaggagttcactgtgcctgggagcaagtctacagctaccatcagcggccttaaacctggagttgattataccatcactgtgtatgctgtcactggcgacggacgtagccccgcaagcagcaagccaatttccattaattaccgaacaggatcccaccatcaccatcatcactga

SEQ ID NO: 14 - protein, 105 aa, Artificial Sequence
  DGR Scrambled monobody
MASVSDVPRDLEVVAATPTSLLISWDAPAVTVRYYRITYGETGGNSPVQEFTVPGSKSTATISGLKPGVDYTITVYAVTGDGRSPASSKPISINYRTGSHHHHHH

SEQ ID NO: 15 - protein, 7 aa, Artificial Sequence
  Int-alpha
KLGFFKR

SEQ ID NO: 16 - protein, 10 aa, Artificial Sequence
  Hep-I
GQPMYGQPMY

SEQ ID NO: 17 - DNA, 31 bp, Artificial Sequence
  Nhe1
tacatatggctagcgtttctgatgttccgag

SEQ ID NO: 18 - DNA, 38 bp, Artificial Sequence
  BamH1
tactgagtggatcctgttcggtaattaatggaaattgg

SEQ ID NO: 19 - DNA, 57 bp, Artificial Sequence
  Rluc8 F
tccattaattaccgaacaggtagcggcagcggtagcgcttccaaggtgtacgacccc

SEQ ID NO: 20 - DNA, 44 bp, Artificial Sequence
  Rluc8 R
tgatgatggtgatggtgggatccctgctcgttcttcagcacgcg

SEQ ID NO: 21 - protein, 6 aa, Artificial Sequence
  tetracystein motif
CCXXCC